European Patent Specification EP 3 508 835 B1, published December 24, 2025. Title: METHOD FOR PREPARING SPECIMEN FOR SKIN ANALYZING OR OBSERVING. Applicant: KABUSHIKI KAISHA YAKULT HONSHA. The sequence listing filed with the application follows.

SEQUENCE LISTING (2 sequences)

SEQ ID NO: 1 - DNA, 22 bp, Artificial Sequence
  synthetic oligonucleotide
gcgtgagtgacggtaatgggta

SEQ ID NO: 2 - DNA, 18 bp, Artificial Sequence
  synthetic oligonucleotide
ttccgacgcgatcaacca